European Patent Application EP 4 417 699 A1, published August 21, 2024. Title: A method for preparation of rebaudioside D and rebaudioside M. Applicant: CJ CheilJedang Corporation. The sequence listing filed with the application follows.

SEQUENCE LISTING (10 sequences)

SEQ ID NO: 1 - protein, 441 aa, unidentified
  REGION 1..441: note = UGT-B
MATLRVLMFPWLAYGHISPFLNIAKQLADRGFLIYLCSTLINLESIIKKIPEKYSESIRFVELHLPELPELPPHYHTTNGLPPHLNHTLHKALKMSKPNFSKILQNLKPDLVIYDILQPWAEHVVNEQNIPAVKILTSGAALFSYFFNFLKNPGVEFPFPAIYLPKVEQVKMREMFEKEPNEEDRLAEGNMQIMLMCTSRTIEAKYLDYCTELSNWKVVPVGPPFQDPITNDVDDMELIDWLGTKDENSTVFVCFGSEYFLSREDMEEVAFGLELSNVNFIWVARFPKGEEQNLEDVLPKGFLERIGERGRVLDKFAPQPRILNHPSTGGFISHCGWNSVMESLDFGVPIIAMPMHNDQPINAKLIVELGVAMEIVRDDDGNIHRGEITETLKDVITGETGEILRGKVRDISKNLKSIREEEMNAAAEELIQLCRNSNKYK

SEQ ID NO: 2 - protein, 441 aa, unidentified
  REGION 1..441: note = UGT-B
MATLKVLMFPFLAYGHISPYLNVAKKLADRGFLIYFCSTPINLKSIIKKIPEKYANSIHLIELHLPELPELPPHYHTTNGLPPNLNHILQKALKMSKPNFSKILQNLKPDLVIYDVLQRWAKHVANEQNIPAVKLLTSGAAVFSYFFNVLKKPGVEFPFPGIYLRKIEQVRLSEMMKELEDDDDDDDLLVDGNMQIMLMSTSRTIEAKYIDFCTALTNWKVVPVGPPVQDLITNDADDMELIDWLGTKDENSTVFVSFGSEYFLSKEDMEEVAFALELSNVNFIWVARFPKGEERNLEDALPKGFLERIGERGRVLDKFAPQPRILNHPSTGGFISHCGWNSAMESIDFGVPIIAMPMHLDQPMNARLIVELGVAVEIVRDDDGKIHRGEIAETLKGVITGKTGGKLRAKVRDISKNLKTIRDEEMDAAAEELIQLCRNSN

SEQ ID NO: 3 - protein, 461 aa, unidentified
  REGION 1..461: note = UGT-B
MDASESESSPLHVVIFPWLAMGHLLPCLELAERLAARGHRVSFVSTPRNLARLPPVRPALASLVHLVALPLPRVAGLPDGAESTSDVPPDKFHLHRVAFDGLAAPFTAFLDAACAGGRRPDWVVADFVHHWVAAVAQARKVPCAMLLPCAAGVAALSGPPPESRAEEHQAVSRSMDAAPRFEAELTTEEFAAEDASGLSIMGRFFMTLKRSKLVALRSSPELEPDAFPLLTRLYGKPAVPLGLLPPPPNGDRSASENSEDVAIIQWLDARPAKSVVYVALGSEAPLRAELLRELAHGLELSGTRFLWVLRNPVNGDADTILPDGFMERTAERGLVAVRWVPQVSILAHGAVGAFLTHCGWGSVVEGLQFGHPLIMLPLAGDQGPNARLMEERKVGVLVPRDEKDGSFTRDGVAGAVRAVVVEEGGRVFADNAKRLQGIVASVECNERCIDLFVQHLRSCRN

SEQ ID NO: 4 - protein, 458 aa, unidentified
  REGION 1..458: note = UGT-A
MENKTETTVRRRRRIILFPVPFQGHINPILQLANVLYSKGFSITIFHTNFNKPKTSNYPHFTFRFILDNDPQDERISNLPTHGPLAGMRIPIINEHGADELRRELELLMLASEEDEEVSCLITDALWYFAQSVADSLNLRRLVLMTSSLFNFHAHVSLPQFDELGYLDPDDKTRLEEQASGFPMLKVKDIKSAYSNWQILKEILGKMIKQTKASSGVIWNSFKELEESELETVIREIPAPSFLIPLPKHLTASSSSLLDHDRTVFQWLDQQPPSSVLYVSFGSTSEVDEKDFLEIARGLVDSKQSFLWVVRPGFVKGSTWVEPLPDGFLGERGRIVKWVPQQEVLAHGAIGAFWTHSGWNSTLESVCEGVPMIFSDFGLDQPLNARYMSDVLKVGVYLENGWERGEIANAIRRVMVDEEGEYIRQNARVLKQKADVSLMKGGSSYESLESLVSYISSL

SEQ ID NO: 5 - protein, 808 aa, unidentified
  REGION 1..808: note = Sucrose synthase
MAAKLARLHSLRERLGATFSSHPNELIALFSRYVNQGKGMLQRHQLLAEFDALIEADKEKYAPFEDILRAAQEAIVLPPWVALAIRPRPGVWDYIRVNVSELAVEELSVSEYLAFKEQLVDGHTNSNFVLELDFEPFNASFPRPSMSKSIGNGVQFLNRHLSSKLFQDKESLYPLLNFLKAHNHKGTTMMLNDRIQSLRGLQSSLRKAEEYLMGIPQDTPYSEFNHRFQELGLEKGWGDCAKRVLDTIHLLLDLLEAPDPANLEKFLGTIPMMFNVVILSPHGYFAQSNVLGYPDTGGQVVYILDQVRALENEMLLRIKQQGLDITPKILIVTRLLPDAVGTTCGQRVEKVIGTEHTDILRVPFRSENGILRKWISRFDVWPFLETYTEDVANEIMREMQAKPDLIIGNYSDGNLVATLLAHKLGVTQCTIAHALEKTKYPNSDIYLDKFDSQYHFSCQFTADLIAMNHTDFIITSTFQEIAGSKDTVGQYESHIAFTLPGLYRVVHGIDVFDPKFNIVSPGADMSVYFPYTEADKRLTAFHPEIEELLYSEVENDEHKFVLKDKNKPIIFSMARLDRVKNMTGLVEMYGKNAHLRDLANLVIVCGDHGNQSKDREEQAEFKKMYGLIDQYKLKGHIRWISAQMNRVRNGELYRYICDTKGVFVQPAFYEAFGLTVIEAMTCGLPTIATCHGGPAEIIVDGVSGLHIDPYHSDKAADILVNFFEKCKQDSTYWDNISQGGLQRIYEKYTWKLYSERLMTLTGVYGFWKYVSNLERRETRRYIEMFYALKYRSLASAVPLAVDGESTSK

SEQ ID NO: 6 - DNA, 1326 bp, unidentified
  misc_feature 1..1326: note = UGT-B
  source 1..1326: mol_type = other DNA
atggcgaccttgcgcgtactgatgtttccctggttggcgtatggtcacatttctccttttctcaacatagccaagcagctcgcggatagaggattcctgatctacctttgtagcacgctgatcaacctcgaaagcatcatcaagaaaatccccgaaaaatactctgagtcaattcgttttgtggagcttcacctgcccgaattgcctgaacttcctcctcattaccacacaaccaatggtctgccgccccatctgaaccacacacttcataaagccctgaaaatgtccaaaccaaacttttccaaaatcctgcagaatctgaaacccgatttggtgatttatgacatattgcagccgtgggccgagcatgtcgtaaatgagcagaatattccggcagtcaagatattaacgtcgggtgcagctctgttttcgtatttcttcaactttctaaaaaatccaggggttgaatttccgtttccggcaatttatctcccgaaagtggagcaagtcaagatgcgagaaatgttcgagaaggaacctaatgaagaggatcgtctcgccgagggcaacatgcagattatgttaatgtgcacctctaggaccattgaggccaagtatctagattattgtactgaactgagcaattggaaagttgttccagttggtccaccgttccaagacccgatcaccaacgacgtggacgacatggagctcattgattggctaggcacaaaggatgagaattcaactgttttcgtctgctttggaagtgagtatttcttgtcacgggaagatatggaagaagtagcgtttggtttggagctgagtaatgtgaatttcatctgggtagcccgctttccgaaaggtgaggagcagaaccttgaggatgtattgccgaaaggttttcttgaaagaattggagagcggggccgtgtgttagacaaatttgcaccacagccacgcattttaaatcatccgtccaccggcggattcataagtcattgtggctggaattcagtgatggagagtttagattttggcgttcctatcatcgccatgcctatgcataacgatcaaccaatcaacgcgaagttgatagtggaattgggggtggcaatggaaattgttcgcgatgatgatgggaatattcaccggggtgaaattacggaaactcttaaagatgtcataacgggggaaacaggggagattttgcgtggcaaagtgcgtgacatcagcaaaaatttgaagtctatccgcgaggaagagatgaacgctgcagctgaagagctgattcagctgtgccggaatagcaataagtacaaatag

SEQ ID NO: 7 - DNA, 1326 bp, unidentified
  misc_feature 1..1326: note = UGT-B
  source 1..1326: mol_type = other DNA
atggctactctgaaagtactgatgtttccgtttttggcttatggccacatttctccctatctgaatgtagccaagaagctcgccgatcggggcttcctgatttacttctgctcaacaccgataaatctgaagagcattatcaaaaaaatccctgaaaaatacgcgaatagcattcatcttatcgagcttcacttaccggagttaccggagttaccccctcattaccatacgacgaatggtctcccgccaaacctcaatcacatccttcagaaagcactgaaaatgtcaaagccaaacttctcgaagatcttacagaacctgaaacctgatctggtgatttatgacgtattgcagcggtgggcgaaacatgtcgccaatgaacagaatatcccagcagttaagctcctgacgagtggtgcagccgtgtttagctattttttcaatgtcttgaaaaagccaggggtcgaatttccattcccgggaatttatctgcgcaaaatcgaacaagtaagactgagtgaaatgatgaaagaactggaggacgacgatgacgatgatgatcttctggtggatggcaatatgcaaataatgttgatgagtacctctcgcaccatcgaagccaaatatatcgatttttgcactgcgttgacgaactggaaagttgttccggttggtcctccggttcaggatctgataaccaacgacgcggacgatatggaacttatcgattggctaggcacaaaagatgagaactcaactgtgtttgtctcctttggtagtgagtatttcctgtccaaggaagatatggaagaagtggcttttgcgttggaattatcgaacgtgaactttatctgggttgccagatttccgaaaggggaagagcgaaatctggaagacgcactgccgaagggatttcttgagcggattggagaaaggggacgtgttttggataaatttgccccccagccacgtattctgaaccatccgtctaccggcggttttatatcccattgtggttggaattcagcaatggaatctatagacttcggggttcctatcatcgcgatgcctatgcacctagatcagcccatgaacgctcgtctcatcgtagaattaggcgttgcggtcgagattgttcgtgatgatgatggtaagatccacagaggagaaatcgcggaaaccttgaaaggtgtgataacagggaaaacaggtggaaagctccgtgctaaagtgcgcgacattagtaaaaacttaaaaaccatacgcgacgaagagatggatgcagctgctgaggagctaatccagctttgtcgcaatagcaattag

SEQ ID NO: 8 - DNA, 1386 bp, unidentified
  misc_feature 1..1386: note = UGT-B
  source 1..1386: mol_type = other DNA
atggatgcgtcggaaagcgagtcatctccgctccacgttgttatatttccttggttagcaatgggtcatctgctcccgtgtctggaactggcagaacgattggcagcacgtggtcatcgggtttcgttcgttagcactcccagaaatttagcacgtttaccaccagttcgtcctgcattggcatcactcgttcatctggttgcactgccgttgcctcgtgttgcaggtctgcccgatggagcagaaagtacatctgatgttccgccggataaatttcaccttcatcgtgttgctttcgatggtttggctgcaccatttaccgcatttctggatgcagcttgcgcaggaggtaggcgtcctgattgggttgtggcagattttgtacatcattgggttgctgcagttgcacaagcacgtaaggtaccgtgtgcaatgttactgccttgcgcagcaggtgttgcagcactaagcggtccaccaccggaaagtcgtgcagaggaacatcaggctgttagtcgaagcatggatgcggcaccacgttttgaagcagaactgactaccgaggaatttgctgcggaagatgcgagtggtctgagtattatgggacgttttttcatgacgctgaaaagatctaaattagttgctctacgttcatcaccggaattagaaccggatgcatttccgctgctgacccgtctttatggtaaaccggcagttccgcttggactgttaccgccccctcctaacggagatagaagcgcaagcgaaaatagcgaggatgttgcaattatccagtggttggatgcacgtccagccaaatctgttgtttacgttgcactgggtagcgaagcacccctccgtgcagaactgttacgtgaattagcacatggacttgaactgtctggtacgcgatttttatgggttctgcgtaatccagttaacggtgatgcagatacgattttacctgatggttttatggaacgtacagcagaacgtggtcttgttgcagttcgttgggtacctcaagtaagcatcctggcacacggtgcagttggtgcattcttaacccactgtgggtggggttcagttgttgaaggtcttcaatttggtcatccattgattatgcttccgcttgcaggcgatcaggggcccaacgctcgcttaatggaagaacgtaaagttggtgttttggtaccccgtgacgaaaaggatggttcgtttacacgtgatggtgttgcaggtgcagttagagcagttgttgttgaagaaggtggtcgtgtatttgcagataatgcaaaacgtctgcagggtatagttgcgagtgttgaatgcaatgagagatgcattgatctgtttgtacagcatctacgtagctgtcgtaattag

SEQ ID NO: 9 - DNA, 1377 bp, unidentified
  misc_feature 1..1377: note = UGT-A
  source 1..1377: mol_type = other DNA
atggaaaataaaacggagaccaccgttcgccggcgccggagaataatattattcccggtaccatttcaaggccacattaacccaattcttcagctagccaatgtgttgtactctaaaggattcagtatcaccatctttcacaccaacttcaacaaacccaaaacatctaattaccctcacttcactttcagattcatcctcgacaacgacccacaagacgaacgcatttccaatctaccgactcatggtccgctcgctggtatgcggattccgattatcaacgaacacggagctgacgaattacgacgcgaactggaactgttgatgttagcttctgaagaagatgaagaggtatcgtgtttaatcacggatgctctttggtacttcgcgcaatctgttgctgacagtcttaacctccgacggcttgttttgatgacaagcagcttgtttaattttcatgcacatgtttcacttcctcagtttgatgagcttggttacctcgatcctgatgacaaaacccgtttggaagaacaagcgagtgggtttcctatgctaaaagtgaaagacatcaagtctgcgtattcgaactggcaaatactcaaagagatattagggaagatgataaaacaaacaaaagcatcttcaggagtcatctggaactcatttaaggaactcgaagagtctgagctcgaaactgttatccgtgagatcccggctccaagtttcttgataccactccccaagcatttgacagcctcttccagcagcttactagaccacgatcgaaccgtttttcaatggttagaccaacaaccgccaagttcggtactgtatgttagttttggtagtactagtgaagtggatgagaaagatttcttggaaatagctcgtgggttggttgatagcaagcagtcgtttttatgggtggttcgacctgggtttgtcaagggttcgacgtgggtcgaaccgttgccagatgggttcttgggtgaaagaggacgtattgtgaaatgggttccacagcaagaagtgctagctcatggagcaataggcgcattctggactcatagcggatggaactctacgttggaaagcgtttgtgaaggtgttcctatgattttctcggattttgggctcgatcaaccgttgaatgctagatacatgagtgatgttttgaaggtaggggtgtatttggaaaatgggtgggaaagaggagagatagcaaatgcaataagaagagttatggtggatgaagaaggagaatacattagacagaatgcaagagttttgaaacaaaaggcagatgtttctttgatgaagggtggttcgtcttacgaatcattagagtctctagtttcttacatttcatcgttgtaa

SEQ ID NO: 10 - DNA, 2427 bp, unidentified
  misc_feature 1..2427: note = Sucrose synthase
  source 1..2427: mol_type = other DNA
atggctgccaagctagctcgcctccacagtctccgcgaacgcctcggtgccaccttctcgtctcatcccaatgagttgattgcactcttctctaggtatgttaaccagggaaagggaatgctccagcgtcaccagctgcttgcggagttcgatgccttgatcgaagctgacaaagagaaatatgctccctttgaagacattctccgggctgctcaggaagccattgtgctgccgccctgggttgcactggccatcaggccaaggcctggtgtctgggactacattcgggtgaatgtaagtgagttggcagtggaagagctgagtgtttctgagtacttggcattcaaggaacagcttgttgatggacacaccaacagcaactttgttcttgagcttgattttgagcccttcaatgcctccttcccgcgcccgtccatgtccaagtccatcggaaatggggtgcagttccttaaccgtcacctgtcgtccaagttgttccaggacaaggagagcctctaccccttgctgaacttcctgaaagcccataaccacaagggcacgacaatgatgctgaatgacagaattcagagccttcgtgggctccaatcatcccttagaaaggcagaagaatatctgatgggcattcctcaagacacgccctactcggagttcaaccacaggttccaagagctcggtttggagaagggttggggtgactgtgcaaagcgtgtgcttgacaccatccacttgcttcttgaccttcttgaggcccctgatccggccaacttggagaagttccttggaactattccaatgatgttcaatgttgttatcctgtctccgcatggatactttgcccaatccaatgtgttgggataccctgatactggtggtcaggttgtgtacattttggaccaagtccgcgctttggagaatgagatgcttttgaggatcaagcagcaaggccttgatatcacacctaagatcctcattgtaaccaggctgttgcctgatgctgttggtactacatgcggccagcgtgtggagaaggttattggaactgagcacactgacattcttcgtgttccattcaggagtgagaatggtatcctccgcaagtggatctcccgttttgatgtctggccattcctggaaacatacactgaggatgttgcaaacgaaattatgagggaaatgcaagccaaacctgatctcatcattggcaattacagtgatggaaaccttgttgccactctgctggctcacaaattaggagttacccagtgtaccattgctcatgccttggagaaaaccaaataccccaactcagacatatacttggacaagtttgacagccagtaccacttctcatgccaattcactgctgatcttatcgccatgaatcacactgatttcatcatcaccagtacattccaagaaattgctggaagcaaggacactgtggggcagtatgaatcacacattgcattcacccttcctgggctttaccgagttgtgcatggcatagatgtttttgatcccaagttcaacattgtctctcctggagctgacatgagtgtctacttcccgtacaccgaggctgacaagaggctcactgctttccaccctgaaattgaggagcttctctacagtgaagtcgagaacgatgaacacaagtttgtattgaaggacaagaacaagccaatcatcttctccatggctcgtcttgaccgagtgaagaacatgacaggtctggttgagatgtatggtaagaatgcacatctcagggatttggcaaaccttgtgattgtttgtggtgaccacggcaatcagtccaaggacagggaggagcaggctgagttcaagaagatgtacggtctcattgaccagtacaagttgaaggggcatatccgctggatctcagctcagatgaaccgtgttcgtaacggggagttgtaccgatacatttgtgacaccaagggagtctttgtccagcctgcattctatgaagcgtttggtctgactgtcatcgaagccatgacatgtggtttgccaacaatcgcaacatgccatggtggccctgctgagattattgttgatggggtgtctggtctgcacattgatccttaccacagtgacaaggctgctgatatcttggtcaacttctttgagaagtgcaagcaggattcaacctactgggacaatatttcacagggaggtctgcagaggatttacgagaagtacacctggaagctgtactctgagaggctgatgaccttgactggtgtatacggattctggaagtacgtaagcaaccttgagaggcgcgagactcgccgttacattgagatgttctatgctctgaaataccgcagcctggccagcgccgtcccattggctgtcgatggagagagcacatccaagtaa